European Patent Application EP 4 141 119 A2, published March 1, 2023. Title: HAIRPIN LOOP ENDED SELF-COMPLEMENTARY DOUBLE-STRANDED COVALENTLY CLOSED LINEAR DNA VECTOR, MANUFACTURING SYSTEM AND PROCESS, AND USES OF SAID RESULTING DNA VECTOR. Applicant: Williams, Mr. Martin. Application EP EP22188491.9, filed August 3, 2022. The sequence listing filed with the application follows.

SEQUENCE LISTING (26 sequences)

SEQ ID NO: 1 - DNA, 5951 bp, synthetic construct
  source 1..5951: mol_type = other DNA
ggatccactagtatctcgacgcattcattaccctgttatccctagatacaagatacattaccctgttatcccagatgacataccctgttatccctagatgacattaccctgttatcccagatgacattaccctgttatccctagatacattaccctgttatcccagatgacataccctgttatccctagatgacattaccctgttatcccagatgacattaccctgttatccctagatacattaccctgttatcccagatgacataccctgttatccctagatgacattaccctgttatcccagatgacattaccctgttatccctagatacattaccctgttatcccagatgacataccctgttatccctagatgacattaccctgttatcccagatgacattaccctgttatccctagatacattaccctgttatcccagatgacataccctgttatccctagatgacattaccctgttatcccagatgacattaccctgttatccctagaagatcctttgatgcggccgcataacttcgtatagcatacattatacgaagttatctcgaggtcagtgtcaagtcagtgactactgtactgaactgtacgatatcggtacctagatgtcaacttcagcacacaattgccattatacgcgcgtataatggactattgtgtgctgatacgatcgcagaccatggtccttcgattggtgtggaaagtccccaggctccccagcaggcagaagtatgcaaagcatgcatctcaattagtcagcaaccagcatgcatgcattggtgtggaaagtccccaggctccccagcaggcagaagtatgcaaagcatgcatctcaattagtcagcaaccagcatgcatgcatctatccatagctgattggtctaaaatgagatacatcaacgctcctccatgttttttgttttctttttaaatgaaaaactttattttttaagaggagtttcaggttcatagcaaaattgagaggaaggtacattcaagctgaggaagttttcctctattcctagtttactgagagattgcatcatgaatgggtgttaaattttgtcaaatgctttttctgtgtctatcaatatgaccatgtgattttcttctttaacctgttgatgggacaaattacgttaattgattttcaaacgttgaaccacccttacatatctggaataaattctacttggttgtggtgtatattttttgatacattcttggattctttttgctaatattttgttgaaaatgtttgtatctttgttcatgagagatattggtctgttgttttcttttcttgtaatgtcattttctagttccggtattaaggtaatgctggcctagttgaatgatttaggaagtattccctctgcttctgtcttctgaaagagattgtagaaagttgatacaatttttttttctttaaatatcttgataggtggctatggcagggcttgccgccccgacgttggctgcgagccctgggccttcacccgaacttgggggttggggtggggaaaaggaagaaacgcgggcgtattggtcccaatggggtctcggtggggtatcgacagagtgccagccctgggaccgaaccccgcgtttatgaacaaacgacccaacacccgtgcgttttattctgtctttttattgccgtcatagcgcgggttccttccggtattgtctccttccgtgtttcagttagcctcccccatctcccgctgcaggaattccgcggaacccctatttgtttatttttctaaatacattcaaatatgtatccgctcatgagacaataaccctgataaatgcttcaataatattgaaaaaggaagagtatgcgtttgaaggtgatgatggatgtcaataaaaaaaccaagattcgtcatcgtaatgagcttaatcataccttagctcagctgcctttaccagcaaaacgcgtgatgtatatggcccttgcccccattgacagtaaggagccgttagaacgcggtcgtgtatttaagattcgtgccgaagacttagcggcgcttgcaaaaattactcctagtttggcctaccgtcaactgaaggagggaggcaaattgctgggcgcctcgaagatcagcttgcgtggagacgatatcatcgcccttgctaaggagttgaacttgccattcactgcgaaaaattccccggaggaattagacctgaatatcattgagtggatcgcttacagccctgacgagggctacttgagtctgaagttcacgcgtactattgagccttatatttctagtcttatcgggaaaaagaacaaatttaccacgcaattattgactgcatccttgcgcctgtcgtcacagtattcttcatcactgtatcaactgatccgcaaacattatagtaatttcaaaaaaaaaaactattttatcattagcgtggacgagcttaaagaagaactgattgcctatacttttgataaagacgggaacatcgaatataaatacccggacttcccaatttttaaacgcgatgttttaaacaaagcgattgcagaaatcaaaaagaaaactgagatttcgtttgttggttttacagtacacgagaaggaggggcgcaaaatttccaaattaaaatttgaatttgtcgttgatgaggacgagtttagtggagataaagacgacgaggctttctttatgaacttgtcggaggccgatgcggcatttttaaaagtgttcgatgaaaccgttccgcccaaaaaagccaagggctaaaagcccgaaaggaagctgagttggctgctgccaccgctgagcaataactagcataaccccttggggcctctaaacgggtcttgaggggttttttggctagctctagagtcgacgatcataatcagccataccacatttgtagaggttttacttgctttaaaaaacctcccacacctccccctgaacctgaaacataaaatgaatgcaattgttgttgttaacttgtttattgcagcttataatggttacaaataaagcaatagcatcacaaatttcacaaataaagcatttttttcactgcattctagttgtggtttgtccaaactcatcaatgtatcttatcatgtctggatcctatccatagctgattggtctaaaatgagatacatcaacgctcctccatgttttttgttttctttttaaatgaaaaactttattttttaagaggagtttcaggttcatagcaaaattgagaggaaggtacattcaagctgaggaagttttcctctattcctagtttactgagagattgcatcatgaatgggtgttaaattttgtcaaatgctttttctgtgtctatcaatatgaccatgtgattttcttctttaacctgttgatgggacaaattacgttaattgattttcaaacgttgaaccacccttacatatctggaataaattctacttggttgtggtgtatattttttgatacattcttggattctttttgctaatattttgttgaaaatgtttgtatctttgttcatgagagatattggtctgttgttttcttttcttgtaatgtcattttctagttccggtattaaggtaatgctggcctagttgaatgatttaggaagtattccctctgcttctgtcttctgaaagagattgtagaaagttgatacaatttttttttctttaaatatcttgataggcacgcatgcattggtgtggaaagtccccaggctccccagcaggcagaagtatgcaaagcatgcatctcaattagtcagcaaccagcatgcatgcattggtgtggaaagtccccaggctccccagcaggcagaagtatgcaaagcatgcatctcaattagtcagcaaccagcatgcatgcatgcgaagtacgagctccgatctccaatttatcagcacacaatagtccattatacgcgcgtataatggcaattgtgtgctgactacgtacgtacactactacgaactcagagtcagtagatctgatatcatcgtctacacttgccagcgccctagcgcccgctcctttcgctttcttcccttcctttctcgccacgttcgccggctttccccgtcaagctctaaatcgggggctccctttagggttccgatttagtgctttacggcacctcgaccccaaaaaacttgatttgggtgatggttcacgtagtgggccatcgccctgatagacggtttttcgccctttgacgttggagtccacgttctttaatagtggactcttgttccaaactggaacaacactcaaccctatctcgggctattcttttgatttataagggattttgccgatttcgggaagatcctttgatggtgccagggcgtgcccttgggctccccgggcgcgcttttctacggggttgacgctcagtcctcgcggaacccctatttgtttatttttctaaatacattcaaatatgtatccgctcatgagacaataaccctgataaatgcttcaataatattgaaaaaggaagagtatgagtattcaacatttccgtgtcgcccttattcccttttttgcggcattttgccttcctgtttttgctcacccagaaacgctggtgaaagtaaaagatgctgaagatcagttgggtgcacgagtgggttacatcgaactggatctcaacagcggtaagatccttgagagttttcgccccgaagaacgttttccaatgatgagcacttttaaagttctgctatgtggcgcggtattatcccgtattgacgccgggcaagagcaactcggtcgccgcatacactattctcagaatgacttggttgagtactcaccagtcacagaaaagcatcttacggatggcatgacagtaagagaattatgcagtgctgccataaccatgagtgataacactgcggccaacttacttctgacaacgatcggaggaccgaaggagctaaccgcttttttgcacaacatgggggatcatgtaactcgccttgatcgttgggaaccggagctgaatgaagccataccaaacgacgagcgtgacaccacgatgcctgtagcaatggcaacaacgttgcgcaaactattaactggcgaactacttactctagcttcccggcaacaattaatagactggatggaggcggataaagttgcaggaccacttctgcgctcggcccttccggctggctggtttattgctgataaatctggagccggtgagcgtgggtctcgcggtatcattgcagcactggggccagatggtaagccctcccgtatcgtagttatctacacgacggggagtcaggcaactatggatgaacgaaatagacagatcgctgagataggtgcctcactgattaagcattggtaactgtcagaccaagtttactcatatatactttagattgatttaaaacttcatttttaatttaaaaggatctaggtgaagatcctttttgataatctcatgaccaaaatcccttaacgtgagttttcgttccactgagcgtcagaccccgtagaaaagatcaaaggatcttccggaccgaaagagtttgtagaaacgcatgtcagccgttaagtgttcctgtgtcactcaaaattgctttgagaggctctaagggcttctcagtgcgttacatccctggcttgttgtccacaaccgttaaaccttaaaagctttaaaagccttatatattcttttttttcttataaaacttaaaaccttagaggctatttaagttgctgatttatattaattttattgttcaaacatgagagcttagtacgtgaaacatgagagcttagtacgttagccatgagagcttagtacgttagccatgagggtttagttcgttaaacatgagagcttagtacgttaaacttgagagcttagtacgtgaaacatgagagcttagtacgtac

SEQ ID NO: 2 - DNA, 73 bp, Artificial
  source 1..73: mol_type = other DNA
  misc_feature 1..73: function = DNA Scaffold Matrix Attachment Region (S/MAR)
tggtgtggaaagtccccaggctccccagcaggcagaagtatgcaaagcatgcatctcaattagtcagcaacca

SEQ ID NO: 3 - DNA, 42 bp, Artificial
  source 1..42: mol_type = other DNA
  misc_feature 1..42: function = DNA Nuclear Localization Sequence
tggggactttccgctggggactttccgctggggactttccgc

SEQ ID NO: 4 - DNA, 2668 bp, Artificial
  source 1..2668: mol_type = other DNA
gggacgtagcagaaggacgtcccgcgcagaatccaggtggcaacacaggcgagcagccaaggaaaggacgatgatttccccgacaacaccacggaattgtcagtgcccaacagccgagcccctgtccagcagcgggcaaggcaggcggcgatgagttccgccgtggcaatagggagggggaaagcgaaagtcccggaaaggagctgacaggtggtggcaatgccccaaccagtgggggttgcgtcagcaaacacagtgcacaccacgccacgttgcctgacaacgggccacaactcctcataaagagacagcaaccaggatttatacaaggaggagaaaatgaaagccatacgggaagcaatagcatgatacaaaggcattaaagcagcgtatccacatagcgtaaaaggagcaacatagttaagaataccagtcaatctttcacaaattttgtaatccagaggttgatctagcagcaaggtcgccacgcacaagatcaatattaacaatcagtcatctctctttagcaataaaaaggtgaaaaattacattttaaaaatgacaccatagacgatgtatgaaaataatctacttggaaataaatctaggcaaagaagtgcaagactgttacccagaaaacttacaaattgtaaatgagaggttagtgaagatttaaatgaatgaagatctaaataaacttataaattgtgagagaaattaatgaatgtctaagttaatgcagaaacggagagacatactatattcatgaactaaaagacttaatattgtgaaggtatactttctttccacataaatttgtagtcaatatgttcaccccaaaaaagctgtttgttaacttgccaacctcattctaaaatgtatatagaagcccaaaagacaataacaaaaatattcttgtagaacaaaatgggaaagaatgttccactaaatatcaagatttagagcaaagcatgagatgtgtggggatagacagtgaggctgataaaatagagtagagctcagaaacagacccattgatatatgtaagtgacctatgaaaaaaatatggcattttacaatgggaaaatgatgatctttttcttttttagaaaaacagggaaatatatttatatgtaaaaaataaaagggaacccatatgtcataccatacacacaaaaaaattccagtgaattataagtctaaatggagaaggcaaaactttaaatcttttagaaaataatatagaagcatgccatcatgacttcagtgtagagaaaaatttcttatgactcaaagtcctaaccacaaagaaaagattgttaattagattgcatgaatattaagacttatttttaaaattaaaaaaccattaagaaaagtcaggccatagaatgacagaaaatatttgcaacaccccagtaaagagaattgtaatatgcagattataaaaagaagtcttacaaatcagtaaaaaataaaactagacaaaaatttgaacagatgaaagagaaactctaaataatcattacacatgagaaactcaatctcagaaatcagagaactatcattgcatatacactaaattagagaaatattaaaaggctaagtaacatctgtggcaatattgatggtatataaccttgatatgatgtgatgagaacagtactttaccccatgggcttcctccccaaacccttaccccagtataaatcatgacaaatatactttaaaaaccattaccctatatctaaccagtactcctcaaaactgtcaaggtcatcaaaaataagaaaagtctgaggaactgtcaaaactaagaggaacccaaggagacatgagaattatatgtaatgtggcattctgaatgagatcccagaacagaaaaagaacagtagctaaaaaactaatgaaatataaataaagtttgaactttagttttttttaaaaaagagtagcattaacacggcaaagccattttcatatttttcttgaacattaagtacaagtctataattaaaaattttttaaatgtagtctggaacattgccagaaacagaagtacaacagctatctgtgctgtcgcctaactatccatagctgattggtctaaaatgagatacatcaacgctcctccatgttttttgttttctttttaaatgaaaaactttattttttaagaggagtttcaggttcatagcaaaattgagaggaaggtacattcaagctgaggaagttttcctctattcctagtttactgagagattgcatcatgaatgggtgttaaattttgtcaaatgctttttctgtgtctatcaatatgaccatgtgattttcttctttaacctgttgatgggacaaattacgttaattgattttcaaacgttgaaccacccttacatatctggaataaattctacttggttgtggtgtatattttttgatacattcttggattctttttgctaatattttgttgaaaatgtttgtatctttgttcatgagagatattggtctgttgttttcttttcttgtaatgtcattttctagttccggtattaaggtaatgctggcctagttgaatgatttaggaagtattccctctgcttctgtcttctgaaagagattgtagaaagttgatacaatttttttttctttaaatatttgatag

SEQ ID NO: 5-10 - skipped (6 entries)

SEQ ID NO: 11 - DNA, 918 bp, Artificial
  source 1..918: mol_type = other DNA
atgcgcctgaaagtgatgatggatgtgaacaaaaaaaccaaaattcgccatcgcaacgaactgaaccataccctggcgcagctgccgctgccggcgaaacgcgtgatgtatatggcgctggcgccgattgatagcaaagaaccgctggaacgcggccgcgtgtttaaaattcgcgcggaagatctggcggcgctggcgaaaattaccccgagcctggcgtatcgccagctgaaagaaggcggcaaactgctgggcgcgagcaaaattagcctgcgcggcgatgatattattgcgctggcgaaagaactgaacctgccgtttaccgcgaaaaacagcccggaagaactggatctgaacattattgaatggattgcgtatagcccggatgaaggctatctgagcctgaaatttacccgcaccattgaaccgtatattagcagcctgattggcaaaaaaaacaaatttaccacccagctgctgaccgcgagcctgcgcctgagcagccagtatagcagcagcctgtatcagctgattcgcaaacattatagcaactttaaaaaaaaaaactattttattattagcgtggatgaactgaaagaagaactgattgcgtatacctttgataaagatggcaacattgaatataaatatccggattttccgatttttaaacgcgatgtgctgaacaaagcgattgcggaaattaaaaaaaaaaccgaaattagctttgtgggctttaccgtgcatgaaaaagaaggccgcaaaattagcaaactgaaatttgaatttgtggtggatgaagatgaatttagcggcgataaagatgatgaagcgttttttatgaacctgagcgaagcggatgcggcgtttctgaaagtgtttgatgaaaccgtgccgccgaaaaaagcgaaaggctaa

SEQ ID NO: 12 - DNA, 179 bp, Artificial
  source 1..179: mol_type = other DNA
tctaaatcgggggctccctttagggttccgatttagtgctttacggcacctcgaccccaaaaaacttgatttgggtgatggttcacgtagtgggccatcgccctgatagacggtttttcgccctttgacgttggagtccacgttctttaatagtggactcttgttccaaactggaacaa

SEQ ID NO: 13 - DNA, 14657 bp, Artificial
  source 1..14657: mol_type = other DNA
tcgcgcgtttcggtgatgacggtgaaaacctctgacacatgcagctcccggagacggtcacagcttgtctgtaagcggatgccgggagcagacaagcccgtcagggcgcgtcagcgggtgttggcgggtgtcggggctggcttaactatgcggcatcagagcagattgtactgagagtgcaccatatgcggtgtgaaataccgcacagatgcgtaaggagaaaataccgcatcaggcgccattcgccattcaggctgcgcaactgttgggaagggcgatcggtgcgggcctcttcgctattacgccagctggcgaaagggggatgtgctgcaaggcgattaagttgggtaacgccagggttttcccagtcacgacgttgtaaaacgacggccagtgaattggagatcggtacttcgcgaatgcgtcgagatgtagtggccaggacccaacgctgcccgaaattggccaggacccaacgctgcccgaaattccgacaccatcgaatggtgcaaaacctttcgcggtatggcatgatagcgcccggaagagagtcaattcagggtggtgaatgtgaaaccagtaacgttatacgatgtcgcagagtatgccggtgtctcttatcagaccgtttcccgcgtggtgaaccaggccagccacgtttctgcgaaaacgcgggaaaaagtggaagcggcgatggcggagctgaattacattcccaaccgcgtggcacaacaactggcgggcaaacagtcgttgctgattggcgttgccacctccagtctggccctgcacgcgccgtcgcaaattgtcgcggcgattaaatctcgcgccgatcaactgggtgccagcgtggtggtgtcgatggtagaacgaagcggcgtcgaagcctgtaaagcggcggtgcacaatcttctcgcgcaacgcgtcagtgggctgatcattaactatccgctggatgaccaggatgccattgctgtggaagctgcctgcactaatgttccggcgttatttcttgatgtctctgaccagacacccatcaacagtattattttctcccatgaagacggtacgcgactgggcgtggagcatctggtcgcattgggtcaccagcaaatcgcgctgttagcgggcccattaagttctgtctcggcgcgtctgcgtctggctggctggcataaatatctcactcgcaatcaaattcagccgatagcggaacgggaaggcgactggagtgccatgtccggttttcaacaaaccatgcaaatgctgaatgagggcatcgttcccactgcgatgctggttgccaacgatcagatggcgctgggcgcaatgcgcgccattaccgagtccgggctgcgcgttggtgcggatatttcggtagtgggatacgacgataccgaagacagctcatgttatatcccgccgttaaccaccatcaaacaggattttcgcctgctggggcaaaccagcgtggaccgcttgctgcaactctctcagggccaggcggtgaagggcaatcagctgttgcccgtctcactggtgaaaagaaaaaccaccctggcgcccaatacgcaaaccgcctctccccgcgcgttggccgattcattaatgcagctggcacgacaggtttcccgactggaaagcgggcagtgagaattcaataattttgtttaactttaagaaggagatatacatatggctgaagcgcaaaatgatcccctgctgccgggatactcgtttaatgcccatctggtggcgggtttaacgccgattgaggccaacggttatctcgatttttttatcgaccgaccgctgggaatgaaaggttatattctcaatctcaccattcgcggtcagggggtggtgaaaaatcagggacgagaatttgtttgccgaccgggtgatattttgctgttcccgccaggagagattcatcactacggtcgtcatccggaggctcgcgaatggtatcaccagtgggtttactttcgtccgcgcgcctactggcatgaatggcttaactggccgtcaatatttgccaatacggggttctttcgcccggatgaagcgcaccagccgcatttcagcgacctgtttgggcaaatcattaacgccgggcaaggggaagggcgctattcggagctgctggcgataaatctgcttgagcaattgttactgcggcgcatggaagcgattaacgagtcgctccatccaccgatggataatcgggtacgcgaggcttgtcagtacatcagcgatcacctggcagacagcaattttgatatcgccagcgtcgcacagcatgtttgcttgtcgccgtcgcgtctgtcacatcttttccgccagcagttagggattagcgtcttaagctggcgcgaggaccaacgtatcagccaggcgaagctgcttttgagcaccacccggatgcctatcgccaccgtcggtcgcaatgttggttttgacgatcaactctatttctcgcgggtatttaaaaaatgcaccggggccagcccgagcgagttccgtgccggttgtgaagaaaaagtgaatgatgtagccgtcaagttgtcataatgtacaaagcttcgccagggttttcccagtcgagctcaataattttgtttaactttaagaaggagatatacatatgagcacaaaaaagaaaccattaacacaagagcagcttgaggacgcacgtcgccttaaagcaatttatgaaaaaaagaaaaatgaacttggcttatcccaggaatctgtcgcagacaagatggggatggggcagtcaggcgttggtgctttatttaatggcatcaatgcattaaatgcttataacgccgcattgcttgcaaaaattctcaaagttagcgttgaagaatttagcccttcaatcgccagagaaatctacgagatgtatgaagcggttagtatgcagccgtcacttagaagtgagtatgagtaccctgttttttctcatgttcaggcagggatgttctcacctgagcttagaacctttaccaaaggtgatgcggagagatgggtaagcacaaccaaaaaagccagtgattctgcattctggcttgaggttgaaggtaattccatgaccgcaccaacaggctccaagccaagctttcctgacggaatgttaattctcgttgaccctgagcaggctgttgagccaggtgatttctgcatagccagacttgggggtgatgagtttaccttcaagaaactgatcagggatagcggtcaggtgtttttacaaccactaaacccacagtacccaatgatcccatgcaatgagagttgttccgttgtggggaaagttatcgctagtcagtggcctgaagagacgtttggctgagcgcaacgcaattaatgtaagttagctcactcattaggcacaattctcatgtttgacagcttatcatcgactgcacggtgcaccaatgcttctggcgtcaggcagccatcggaagctgtggtatggctgtgcaggtcgtaaatcactgcataattcgtgtcgctcaaggcgcactcccgttctggataatgttttttgcgccgacatcataacggttctggcaaatattctgaaatgagctacggcctcaacctactactgggctgcttcctaatgcaggatttacactttatgcttccggctcgtatgttgtgtggaattgtgagcggataacaatttcacacatactagagtcacacaggaaagtactaggtggacacgtacgcgggtgcttacgaccgtcagtcgcgcgagcgcgagaattcgagcgcagcaagcccagcgacacagcgtagcgccaacgaagacaaggcggccgaccttcagcgcgaagtcgagcgcgacgggggccggttcaggttcgtcgggcatttcagcgaagcgccgggcacgtcggcgttcgggacggcggagcgcccggagttcgaacgcatcctgaacgaatgccgcgccgggcggctcaacatgatcattgtctatgacgtgtcgcgcttctcgcgcctgaaggtcatggacgcgattccgattgtctcggaattgctcgccctgggcgtgacgattgtttccactcaggaaggcgtcttccggcagggaaacgtcatggacctgattcacctgattatgcggctcgacgcgtcgcacaaagaatcttcgctgaagtcggcgaagattctcgacacgaagaaccttcagcgcgaattgggcgggtacgtcggcgggaaggcgccttacggcttcgagcttgtttcggagacgaaggagatcacgcgcaacggccgaatggtcaatgtcgtcatcaacaagcttgcgcactcgaccactccccttaccggacccttcgagttcgagcccgacgtaatccggtggtggtggcgtgagatcaagacgcacaaacaccttcccttcaagccgggcagtcaagccgccattcacccgggcagcatcacggggctttgtaagcgcatggacgctgacgccgtgccgacccggggcgagacgattgggaagaagaccgcttcaagcgcctgggacccggcaaccgttatgcgaatccttcgggacccgcgtattgcgggcttcgccgctgaggtgatctacaagaagaagccggacggcacgccgaccacgaagattgagggttaccgcattcagcgcgacccgatcacgctccggccggtcgagcttgattgcggaccgatcatcgagcccgctgagtggtatgagcttcaggcgtggttggacggcagggggcgcggcaaggggctttcccgggggcaagccattctgtccgccatggacaagctgtactgcgagtgtggcgccgtcatgacttcgaagcgcggggaagaatcgatcaaggactcttaccgctgccgtcgccggaaggtggtcgacccgtccgcacctgggcagcacgaaggcacgtgcaacgtcagcatggcggcactcgacaagttcgttgcggaacgcatcttcaacaagatcaggcacgccgaaggcgacgaagagacgttggcgcttctgtgggaagccgcccgacgcttcggcaagctcactgaggcgcctgagaagagcggcgaacgggcgaaccttgttgcggagcgcgccgacgccctgaacgcccttgaagagctgtacgaagaccgcgcggcaggcgcgtacgacggacccgttggcaggaagcacttccggaagcaacaggcagcgctgacgctccggcagcaaggggcggaagagcggcttgccgaacttgaagccgccgaagccccgaagcttccccttgaccaatggttccccgaagacgccgacgctgacccgaccggccctaagtcgtggtgggggcgcgcgtcagtagacgacaagcgcgtgttcgtcgggctcttcgtagacaagatcgttgtcacgaagtcgactacgggcagggggcagggaacgcccatcgagaagcgcgcttcgatcacgtgggcgaagccgccgaccgacgacgacgaagacgacgcccaggacggcacggaagacgtagcggcgtagttaacctaggctgctgccaccgctgagcaataactagcataaccccttggggcctctaaacgggtcttgaggggttttttgatggtggcaggccccgtggccgggggactgttgggcgccatctcctacttttcatactcccgccattcagagaagaaaccaattgtccatattgcatcagacattgccgtcactgcgtcttttactggctcttctcgctaaccaaaccggtaaccccgcttattaaaagcattctgtaacaaagcgggaccaaagccatgacaaaaacgcgtaacaaaagtgtctataatcacggcagaaaagtccacattgattatttgcacggcgtcacactttgctatgccatagcatttttatccataagattagcggatcctacctgacgctttttatcgcaactctctactgtttctccatacccgtttttttgggctagcgaattcgagctcaagaggataccatatgaaaaacattaaaaaaaaccaggtgatgaacctgggcccgaacagcaaactgctgaaagaatataaaagccagctgattgaactgaacattgaacagtttgaagcgggcattggcctgattctgggcgatgcgtatattcgcagccgcgatgaaggcaaaacctattgcatgcagtttgaatggaaaaacaaagcgtatatggatcatgtgtgcctgctgtatgatcagtgggtgctgagcccgccgcataaaaaagaacgcgtgaaccatctgggcaacctggtgattacctggggcgcgcagacctttaaacatcaggcgtttaacaaactggcgaacctgtttattgtgaacaacaaaaaaaccattccgaacaacctggtggaaaactatctgaccccgatgagcctggcgtattggtttatggatgatggcggcaaatgggattataacaaaaacagcaccaacaaaagcattgtgctgaacacccagagctttacctttgaagaagtggaatatctggtgaaaggcctgcgcaacaaatttcagctgaactgctatgtgaaaattaacaaaaacaaaccgattatttatattgatagcatgagctatctgattttttataacctgattaaaccgtatctgattccgcagatgatgtataaactgccgaacaccattagcagcgaaacctttctgaaatgagaattcaataattttgtttaactttaagaaggagatatacatatgattgacatgctagttttacgattaccgttcatcgattctcttgtttgctccagactctcaggcaatgacctgatagcctttgtagatctctcaaaaatagctaccctctccggcattaatttatcagctagaacggttgaatatcatattgatggtgatttgactgtctccggcctttctcacccttttgaatctttacctacacattactcaggcattgcatttaaaatatatgagggttctaaaaatttttatccttgcgttgaaataaaggcttctcccgcaaaagtattacagggtcataatgtttttggtacaaccgatttagctttatgctctgaggctttattgcttaattttgctaattctttgccttgcctgtatgatttattggatgttaatgctactactattagtagaattgatgccaccttttcagctcgcgccccaaatgaaaatatagctaaacaggttattgaccatttgcgaaatgtatctaatggtcaaactaaatctactcgttcgcagaattgggaatcaactgttatatggaatgaaacttccagacaccgtactttagttgcatatttaaaacatgttgagctacagcattatattcagcaattaagctctaagccatccgcaaaaatgacctcttatcaaaaggagcaattaaaggtactctctaatcctgacctgttggagtttgcttccggtctggttcgctttgaagctcgaattaaaacgcgatatttgaagtctttcgggcttcctcttaatctttttgatgcaatccgctttgcttctgactataatagtcagggtaaagacctgatttttgatttatggtcattctcgttttctgaactgtttaaagcatttgagggggattcaatgaatatttatgacgattccgcagtattggacgctatccagtctaaacattttactattaccccctctggcaaaacttcttttgcaaaagcctctcgctattttggtttttatcgtcgtctggtaaacgagggttatgatagtgttgctcttactatgcctcgtaattccttttggcgttatgtatctgcattagttgaatgtggtattcctaaatctcaactgatgaatctttctacctgtaataatgttgttccgttagttcgttttattaacgtagatttttcttcccaacgtcctgactggtataatgagccagttcttaaaatcgcataatctagagtcgacctgcaggcatgcaagcttggctgttttggcggatgagagaagattttcagcctgatacagattaaatcagaacgcagaagcggtctgataaaacagaatttgcctggcggcagtagcgcggtggtcccacctgaccccatgccgaactcagaagtgaaacgccgtagcgccgatggtagtgtggggtctccccatgcgagagtagggaactgccaggcatcaaataaaacgaaaggctcagtcgaaagactgggcctttcgttttatctgttgtttgtcggtgaacgctctcctgagtaggacaaatccgccgggagcggatttgaacgttgcgaagcaacggcccggagggtggcgggcaggacgcccgccataaactgccaggcatcaaattaagcagaaggccatcctgacggatggcctttttgcgtttctacaaactcgtggccggcatcaccggcgccacaggtgcggttgctgtctcacctaccaaacaatgcccccctgcaaaaaataaattcatataaaaaacatacagataaccatctgcggtgataaattatctctggcggtgttgacataaataccactggcggtgatactgagcacatcagcaggacgcactgaccaccatgaaggtgacgctcttaaaaattaagccctgaagaagggcagcattcaaagcagaaggctttggggtgtgtgatacgaaacgaagcattggccgtaagtgcgattccggattagctgccaatgtgccaatcgcggggggttttcgttcaggactacaactgccacacaccaccaaagctaactgacaggagaatccagatgagcaaggtaaaaatcggtgagttgatcaacacgcttgtgaatgaggtagaggcaattgatgcctcagaccgcccacaaggcgacaaaacgaagagaattaaagccgcagccgcacggtataagaacgcgttatttaatgataaaagaaagttccgtgggaaaggattgcagaaaagaataaccgcgaatacttttaacgcctatatgagcagggcaagaaagcggtttgatgataaattacatcatagctttgataaaaatattaataaattatcggaaaagtatcctctttacagcgaagaattatcttcatggctttctatgcctacggctaatattcgccagcacatgtcatcgttacaatctaaattgaaagaaataatgccgcttgccgaagagttatcaaatgtaagaataggctctaaaggcagtgatgcaaaaatagcaagactaataaaaaaatatccagattggagttttgctcttagtgatttaaacagtgatgattggaaggagcgccgtgactatctttataagttattccaacaaggctctgcgttgttagaagaactacaccagctcaaggtcaaccatgaggttctgtaccatctgcagctaagccctgcggagcgtacatctatacagcaacgatgggccgatgttctgcgcgagaagaagcgtaatgttgtggttattgactacccaacatacatgcagtctatctatgatattttgaataatcctgcgactttatttagtttaaacactcgttctggaatggcacctttggcctttgctctggctgcggtatcagggcgaagaatgattgagataatgtttcagggtgaatttgccgtttcaggaaagtatacggttaatttctcagggcaagctaaaaaacgctctgaagataaaagcgtaaccagaacgatttatactttatgcgaagcaaaattattcgttgaattattaacagaattgcgttcttgctctgctgcatctgatttcgatgaggttgttaaaggatatggaaaggatgatacaaggtctgagaacggcaggataaatgctattttagcaaaagcatttaacccttgggttaaatcatttttcggcgatgaccgtcgtgtttataaagatagccgcgctatttacgctcgcatcgcttatgagatgttcttccgcgtcgatccacggtggaaaaacgtcgacgaggatgtgttcttcatggagattctcggacacgacgatgagaacacccagctgcactataagcagttcaagctggccaacttctccagaacctggcgacctgaagttggggatgaaaacaccaggctggtggctctgcagaaactggacgatgaaatgccaggctttgccagaggtgacgctggcgtccgtctccatgaaaccgttaagcagctggtggagcaggacccatcagcaaaaataaccaacagcactctccgggcctttaaatttagcccgacgatgattagccggtacctggagtttgccgctgatgcattggggcagttcgttggcgagaacgggcagtggcagctgaagatagagacacctgcaatcgtcctgcctgatgaagaatccgttgagaccatcgacgaaccggatgatgagtcccaagacgacgagctggatgaagatgaaattgagctcgacgagggtggcggcgatgaaccaaccgaagaggaagggccagaagaacatcagccaactgctctaaaacccgtcttcaagcctgcaaaaaataacggggacggaacgtacaagatagagtttgaatacgatggaaagcattatgcctggtccggccccgccgatagccctatggccgcaatgcgatccgcatgggaaacgtactacagctaattaacctaggctgctgccaccgctgagcaataaattctcaccaataaaaaacgcccggcggcaaccgagcgttctgaacaaatccagatggagttctgaggtcattactggatctatcaacaggagtccactcaaaggcggtaatacggttattacatcggatgccgggaccgacgagtgcagaggcgtgcaagcgagcttggcgtaatcatggtcatagctgtttcctgtgtgaaattgttatccgctcacaattccacacaacatacgagccggaagcataaagtgtaaagcctggggtgcctaatgagtgagctaactcacattaattgcgttgcgctcactgcccgctttccagtcgggaaacctgtcgtgccagctgcattaatgaatcggccaacgcgcggggagaggcggtttgcgtattgggcgctcttccgcttcctcgctcactgactcgcggccgcgctgcgctcggtcgttcggctgcggcgagcggtagggataacagggtaatgtcatctgggataacagggtaatgtcatctagggataacagggtatgtcatctgggataacagggtaatgtatctagggataacagggtaatgtcatctgggataacagggtaatgtcatctagggataacagggtatgtcatctgggataacagggtaatgtatctagggataacagggtaatgtcatctgggataacagggtaatgtcatctagggataacagggtatgtcatctgggataacagggtaatgtatctagggataacagggtaatgtcatctgggataacagggtaatgtcatctagggataacagggtatgtcatctgggataacagggtaatgtatctagggataacagggtaatgtcatctgggataacagggtaatgtcatctagggataacagggtatgtcatctgggataacagggtaatgtatcttgtatctagggataacagggtaattatcagctcactcaaaggcggtaatacggttatccacagaatcaggggataacgcaggaaagaacatgtgagcaaaaggccagcaaaaggccaggaaccgtaaaaaggccgcgttgctggcgttatggaatagactggatggaggcggataaagttgcaggaccacttctgcgctcggcccttccggctggctggtttattgctgataaatctggagccggtgagcgtgggtctcgcggtatcattgcagcactggggccagatggtaagccctcccgtatcgtagttatctacacgacggggagtcaggcaactatggatgaacgaaatagacagatcgctgagataggtgcctcactgattaagcattggtaactgtcagaccaagtttactcatatatactttagattgatttaaaacttcatttttaatttaaaaggatctaggtgaagatcctttttgataatctcatgaccaaaatcccttaacgtgagttttcgttccactgagcgtcagaccccttaataagatgatcttcttgagatcgttttggtctgcgcgtaatctcttgctctgaaaacgaaaaaaccgccttgcagggcggtttttcgaaggttctctgagctaccaactctttgaaccgaggtaactggcttggaggagcgcagtcaccaaaacttgtcctttcagtttagccttaaccggcgcatgacttcaagactaactcctctaaatcaattaccagtggctgctgccagtggtgcttttgcatgtctttccgggttggactcaagacgatagttaccggataaggcgcagcggtcggactgaacggggggttcgtgcatacagtccagcttggagcgaactgcctacccggaactgagtgtcaggcgtggaatgagacaaacgcggccataacagcggaatgacaccggtaaaccgaaaggcaggaacaggagagcgcacgagggagccgccaggggaaacgcctggtatctttatagtcctgtcgggtttcgccaccactgatttgagcgtcagatttcgtgatgcttgtcaggggggcggagcctatggaaaaacggctttgccgcggccctctcacttccctgttaagtatcttcctggcatcttccaggaaatctccgccccgttcgtaagccatttccgctcgccgcagtcgaacgaccgagcgtagcgagtcagtgagcgaggaagcggaatatatcctgtatcacatattctgctgacgcaccggtgcagccttttttctcctgccacatgaagcacttcactgacaccctcatcagtgccaacatagtaagccagtatacactccgctagcgctgaggtctgcctcgtgaagaaggtgttgctgactcataccaggcctgaatcgccccatcatccagccagaaagtgagggagccacggttgatgagagctttgttgtaggtggaccagttggtgattttgaacttttgctttgccacggaacggtctgcgttgtcgggaagatgcgtgatctgatccttcaactcagcaaaagttcgatttattcaacaaagccacgttgtgtctcaaaatctctgatgttacattgcacaagataaaaatatatcatcatgaacaataaaactgtctgcttacataaacagtaatacaaggggtgttgaagatcctttgagcggccgctcttttctacggggtctgacgctcagtggaacgaaaactcacgttaagggattttggtcatgagattatcaaaaaggatcttcacctagatccttttaaattaaaaatgaagttttaaatcaatctaaagtatatatgagtaaacttggtctgacagttaccaatgcttaatcagtgaggcacctatctcagcgatctgtctatttcgttcatccatagttgcctgactccccgtcgtgtagataactacgatacgggagggcttaccatctggccccagtgctgcaatgataccgcgagacccacgctcaccggctccagatttatcagcaataaaccagccagccggaagggccgagcgcagaagtggtcctgcaactttatccgcctccatccagtctattaattgttgccgggaagctagagtaagtagttcgccagttaatagtttgcgcaacgttgttgccattgctacaggcatcgtggtgtcacgctcgtcgtttggtatggcttcattcagctccggttcccaacgatcaaggcgagttacatgatcccccatgttgtgcaaaaaagcggttagctccttcggtcctccgatcgttgtcagaagtaagttggccgcagtgttatcactcatggttatggcagcactgcataattctcttactgtcatgccatccgtaagatgcttttctgtgactggtgagtactcaaccaagtcattctgagaatagtgtatgcggcgaccgagttgctcttgcccggcgtcaatacgggataataccgcgccacatagcagaactttaaaagtgctcatcattggaaaacgttcttcggggcgaaaactctcaaggatcttaccgctgttgagatccagttcgatgtaacccactcgtgcacccaactgatcttcagcatcttttactttcaccagcgtttctgggtgagcaaaaacaggaaggcaaaatgccgcaaaaaagggaataagggcgacacggaaatgttgaatactcatactcttcctttttcaatattattgaagcatttatcagggttattgtctcatgagcggatacatatttgaatgtatttagaaaaataaacaaataggggttccgcgcacatttccccgaaaagtgccacctgacgtctaagaaaccattattatcatgacattaacctataaaaataggcgtatcacgaggccctttcgtc

SEQ ID NO: 14 - DNA, 29 bp, Artificial
  source 1..29: mol_type = other DNA
ttgacaattaatcatcggctcgtataatg

SEQ ID NO: 15 - DNA, 1083 bp, Artificial
  source 1..1083: mol_type = other DNA
atgaaaccagtaacgttatacgatgtcgcagagtatgccggtgtctcttatcagaccgtttcccgcgtggtgaaccaggccagccacgtttctgcgaaaacgcgggaaaaagtggaagcggcgatggcggagctgaattacattcccaaccgcgtggcacaacaactggcgggcaaacagtcgttgctgattggcgttgccacctccagtctggccctgcacgcgccgtcgcaaattgtcgcggcgattaaatctcgcgccgatcaactgggtgccagcgtggtggtgtcgatggtagaacgaagcggcgtcgaagcctgtaaagcggcggtgcacaatcttctcgcgcaacgcgtcagtgggctgatcattaactatccgctggatgaccaggatgccattgctgtggaagctgcctgcactaatgttccggcgttatttcttgatgtctctgaccagacacccatcaacagtattattttctcccatgaagacggtacgcgactgggcgtggagcatctggtcgcattgggtcaccagcaaatcgcgctgttagcgggcccattaagttctgtctcggcgcgtctgcgtctggctggctggcataaatatctcactcgcaatcaaattcagccgatagcggaacgggaaggcgactggagtgccatgtccggttttcaacaaaccatgcaaatgctgaatgagggcatcgttcccactgcgatgctggttgccaacgatcagatggcgctgggcgcaatgcgcgccattaccgagtccgggctgcgcgttggtgcggatatctcggtagtgggatacgacgataccgaagacagctcatgttatatcccgccgtcaaccaccatcaaacaggattttcgcctgctggggcaaaccagcgtggaccgcttgctgcaactctctcagggccaggcggtgaagggcaatcagctgttgcccgtctcactggtgaaaagaaaaaccaccctggcgcccaatacgcaaaccgcctctccccgcgcgttggccgattcattaatgcagctggcacgacaggtttcccgactggaaagcgggcagtga

SEQ ID NO: 16 - DNA, 879 bp, Artificial
  source 1..879: mol_type = other DNA
atggctgaagcgcaaaatgatcccctgctgccgggatactcgtttaatgcccatctggtggcgggtttaacgccgattgaggccaacggttatctcgatttttttatcgaccgaccgctgggaatgaaaggttatattctcaatctcaccattcgcggtcagggggtggtgaaaaatcagggacgagaatttgtttgccgaccgggtgatattttgctgttcccgccaggagagattcatcactacggtcgtcatccggaggctcgcgaatggtatcaccagtgggtttactttcgtccgcgcgcctactggcatgaatggcttaactggccgtcaatatttgccaatacggggttctttcgcccggatgaagcgcaccagccgcatttcagcgacctgtttgggcaaatcattaacgccgggcaaggggaagggcgctattcggagctgctggcgataaatctgcttgagcaattgttactgcggcgcatggaagcgattaacgagtcgctccatccaccgatggataatcgggtacgcgaggcttgtcagtacatcagcgatcacctggcagacagcaattttgatatcgccagcgtcgcacagcatgtttgcttgtcgccgtcgcgtctgtcacatcttttccgccagcagttagggattagcgtcttaagctggcgcgaggaccaacgtatcagccaggcgaagctgcttttgagcaccacccggatgcctatcgccaccgtcggtcgcaatgttggttttgacgatcaactctatttctcgcgggtatttaaaaaatgcaccggggccagcccgagcgagttccgtgccggttgtgaagaaaaagtgaatgatgtagccgtcaagttgtcataa

SEQ ID NO: 17 - DNA, 714 bp, Artificial
  source 1..714: mol_type = other DNA
atgagcacaaaaaagaaaccattaacacaagagcagcttgaggacgcacgtcgccttaaagcaatttatgaaaaaaagaaaaatgaacttggcttatcccaggaatctgtcgcagacaagatggggatggggcagtcaggcgttggtgctttatttaatggcatcaatgcattaaatgcttataacgccgcattgcttgcaaaaattctcaaagttagcgttgaagaatttagcccttcaatcgccagagaaatctacgagatgtatgaagcggttagtatgcagccgtcacttagaagtgagtatgagtaccctgttttttctcatgttcaggcagggatgttctcacctgagcttagaacctttaccaaaggtgatgcggagagatgggtaagcacaaccaaaaaagccagtgattctgcattctggcttgaggttgaaggtaattccatgaccgcaccaacaggctccaagccaagctttcctgacggaatgttaattctcgttgaccctgagcaggctgttgagccaggtgatttctgcatagccagacttgggggtgatgagtttaccttcaagaaactgatcagggatagcggtcaggtgtttttacaaccactaaacccacagtacccaatgatcccatgcaatgagagttgttccgttgtggggaaagttatcgctagtcagtggcctgaagagacgtttggctga

SEQ ID NO: 18 - DNA, 1233 bp, Artificial
  source 1..1233: mol_type = other DNA
atgattgacatgctagttttacgattaccgttcatcgattctcttgtttgctccagactctcaggcaatgacctgatagcctttgtagatctctcaaaaatagctaccctctccggcattaatttatcagctagaacggttgaatatcatattgatggtgatttgactgtctccggcctttctcacccttttgaatctttacctacacattactcaggcattgcatttaaaatatatgagggttctaaaaatttttatccttgcgttgaaataaaggcttctcccgcaaaagtattacagggtcataatgtttttggtacaaccgatttagctttatgctctgaggctttattgcttaattttgctaattctttgccttgcctgtatgatttattggatgttaatgctactactattagtagaattgatgccaccttttcagctcgcgccccaaatgaaaatatagctaaacaggttattgaccatttgcgaaatgtatctaatggtcaaactaaatctactcgttcgcagaattgggaatcaactgttatatggaatgaaacttccagacaccgtactttagttgcatatttaaaacatgttgagctacagcattatattcagcaattaagctctaagccatccgcaaaaatgacctcttatcaaaaggagcaattaaaggtactctctaatcctgacctgttggagtttgcttccggtctggttcgctttgaagctcgaattaaaacgcgatatttgaagtctttcgggcttcctcttaatctttttgatgcaatccgctttgcttctgactataatagtcagggtaaagacctgatttttgatttatggtcattctcgttttctgaactgtttaaagcatttgagggggattcaatgaatatttatgacgattccgcagtattggacgctatccagtctaaacattttactattaccccctctggcaaaacttcttttgcaaaagcctctcgctattttggtttttatcgtcgtctggtaaacgagggttatgatagtgttgctcttactatgcctcgtaattccttttggcgttatgtatctgcattagttgaatgtggtattcctaaatctcaactgatgaatctttctacctgtaataatgttgttccgttagttcgttttattaacgtagatttttcttcccaacgtcctgactggtataatgagccagttcttaaaatcgcataa

SEQ ID NO: 19 - DNA, 1896 bp, Artificial
  source 1..1896: mol_type = other DNA
atgagcaaggtaaaaatcggtgagttgatcaacacgcttgtgaatgaggtagaggcaattgatgcctcagaccgcccacaaggcgacaaaacgaagagaattaaagccgcagccgcacggtataagaacgcgttatttaatgataaaagaaagttccgtgggaaaggattgcagaaaagaataaccgcgaatacttttaacgcctatatgagcagggcaagaaagcggtttgatgataaattacatcatagctttgataaaaatattaataaattatcggaaaagtatcctctttacagcgaagaattatcttcatggctttctatgcctacggctaatattcgccagcacatgtcatcgttacaatctaaattgaaagaaataatgccgcttgccgaagagttatcaaatgtaagaataggctctaaaggcagtgatgcaaaaatagcaagactaataaaaaaatatccagattggagttttgctcttagtgatttaaacagtgatgattggaaggagcgccgtgactatctttataagttattccaacaaggctctgcgttgttagaagaactacaccagctcaaggtcaaccatgaggttctgtaccatctgcagctaagccctgcggagcgtacatctatacagcaacgatgggccgatgttctgcgcgagaagaagcgtaatgttgtggttattgactacccaacatacatgcagtctatctatgatattttgaataatcctgcgactttatttagtttaaacactcgttctggaatggcacctttggcctttgctctggctgcggtatcagggcgaagaatgattgagataatgtttcagggtgaatttgccgtttcaggaaagtatacggttaatttctcagggcaagctaaaaaacgctctgaagataaaagcgtaaccagaacgatttatactttatgcgaagcaaaattattcgttgaattattaacagaattgcgttcttgctctgctgcatctgatttcgatgaggttgttaaaggatatggaaaggatgatacaaggtctgagaacggcaggataaatgctattttagcaaaagcatttaacccttgggttaaatcatttttcggcgatgaccgtcgtgtttataaagatagccgcgctatttacgctcgcatcgcttatgagatgttcttccgcgtcgatccacggtggaaaaacgtcgacgaggatgtgttcttcatggagattctcggacacgacgatgagaacacccagctgcactataagcagttcaagctggccaacttctccagaacctggcgacctgaagttggggatgaaaacaccaggctggtggctctgcagaaactggacgatgaaatgccaggctttgccagaggtgacgctggcgtccgtctccatgaaaccgttaagcagctggtggagcaggacccatcagcaaaaataaccaacagcactctccgggcctttaaatttagcccgacgatgattagccggtacctggagtttgccgctgatgcattggggcagttcgttggcgagaacgggcagtggcagctgaagatagagacacctgcaatcgtcctgcctgatgaagaatccgttgagaccatcgacgaaccggatgatgagtcccaagacgacgagctggatgaagatgaaattgagctcgacgagggtggcggcgatgaaccaaccgaagaggaagggccagaagaacatcagccaactgctctaaaacccgtcttcaagcctgcaaaaaataacggggacggaacgtacaagatagagtttgaatacgatggaaagcattatgcctggtccggccccgccgatagccctatggccgcaatgcgatccgcatgggaaacgtactacagctaa

SEQ ID NO: 20 - DNA, 1818 bp, Artificial
  source 1..1818: mol_type = other DNA
atggacacgtacgcgggtgcttacgaccgtcagtcgcgcgagcgcgagaattcgagcgcagcaagcccagcgacacagcgtagcgccaacgaagacaaggcggccgaccttcagcgcgaagtcgagcgcgacgggggccggttcaggttcgtcgggcatttcagcgaagcgccgggcacgtcggcgttcgggacggcggagcgcccggagttcgaacgcatcctgaacgaatgccgcgccgggcggctcaacatgatcattgtctatgacgtgtcgcgcttctcgcgcctgaaggtcatggacgcgattccgattgtctcggaattgctcgccctgggcgtgacgattgtttccactcaggaaggcgtcttccggcagggaaacgtcatggacctgattcacctgattatgcggctcgacgcgtcgcacaaagaatcttcgctgaagtcggcgaagattctcgacacgaagaaccttcagcgcgaattgggcgggtacgtcggcgggaaggcgccttacggcttcgagcttgtttcggagacgaaggagatcacgcgcaacggccgaatggtcaatgtcgtcatcaacaagcttgcgcactcgaccactccccttaccggacccttcgagttcgagcccgacgtaatccggtggtggtggcgtgagatcaagacgcacaaacaccttcccttcaagccgggcagtcaagccgccattcacccgggcagcatcacggggctttgtaagcgcatggacgctgacgccgtgccgacccggggcgagacgattgggaagaagaccgcttcaagcgcctgggacccggcaaccgttatgcgaatccttcgggacccgcgtattgcgggcttcgccgctgaggtgatctacaagaagaagccggacggcacgccgaccacgaagattgagggttaccgcattcagcgcgacccgatcacgctccggccggtcgagcttgattgcggaccgatcatcgagcccgctgagtggtatgagcttcaggcgtggttggacggcagggggcgcggcaaggggctttcccgggggcaagccattctgtccgccatggacaagctgtactgcgagtgtggcgccgtcatgacttcgaagcgcggggaagaatcgatcaaggactcttaccgctgccgtcgccggaaggtggtcgacccgtccgcacctgggcagcacgaaggcacgtgcaacgtcagcatggcggcactcgacaagttcgttgcggaacgcatcttcaacaagatcaggcacgccgaaggcgacgaagagacgttggcgcttctgtgggaagccgcccgacgcttcggcaagctcactgaggcgcctgagaagagcggcgaacgggcgaaccttgttgcggagcgcgccgacgccctgaacgcccttgaagagctgtacgaagaccgcgcggcaggcgcgtacgacggacccgttggcaggaagcacttccggaagcaacaggcagcgctgacgctccggcagcaaggggcggaagagcggcttgccgaacttgaagccgccgaagccccgaagcttccccttgaccaatggttccccgaagacgccgacgctgacccgaccggccctaagtcgtggtgggggcgcgcgtcagtagacgacaagcgcgtgttcgtcgggctcttcgtagacaagatcgttgtcacgaagtcgactacgggcagggggcagggaacgcccatcgagaagcgcgcttcgatcacgtgggcgaagccgccgaccgacgacgacgaagacgacgcccaggacggcacggaagacgtagcggcgtag

SEQ ID NO: 21 - DNA, 708 bp, Artificial
  source 1..708: mol_type = other DNA
atgaaaaacattaaaaaaaaccaggtgatgaacctgggcccgaacagcaaactgctgaaagaatataaaagccagctgattgaactgaacattgaacagtttgaagcgggcattggcctgattctgggcgatgcgtatattcgcagccgcgatgaaggcaaaacctattgcatgcagtttgaatggaaaaacaaagcgtatatggatcatgtgtgcctgctgtatgatcagtgggtgctgagcccgccgcataaaaaagaacgcgtgaaccatctgggcaacctggtgattacctggggcgcgcagacctttaaacatcaggcgtttaacaaactggcgaacctgtttattgtgaacaacaaaaaaaccattccgaacaacctggtggaaaactatctgaccccgatgagcctggcgtattggtttatggatgatggcggcaaatgggattataacaaaaacagcaccaacaaaagcattgtgctgaacacccagagctttacctttgaagaagtggaatatctggtgaaaggcctgcgcaacaaatttcagctgaactgctatgtgaaaattaacaaaaacaaaccgattatttatattgatagcatgagctatctgattttttataacctgattaaaccgtatctgattccgcagatgatgtataaactgccgaacaccattagcagcgaaacctttctgaaatga

SEQ ID NO: 22 - DNA, 357 bp, Artificial
  source 1..357: mol_type = other DNA
tgtcagccgttaagtgttcctgtgtcactcaaaattgctttgagaggctctaagggcttctcagtgcgttacatccctggcttgttgtccacaaccgttaaaccttaaaagctttaaaagccttatatattcttttttttcttataaaacttaaaaccttagaggctatttaagttgctgatttatattaattttattgttcaaacatgagagcttagtacgtgaaacatgagagcttagtacgttagccatgagagcttagtacgttagccatgagggtttagttcgttaaacatgagagcttagtacgttaaacttgagagcttagtacgtgaaacatgagagcttagtacgtac

SEQ ID NO: 23 - DNA, 1136 bp, Artificial
  source 1..1136: mol_type = other DNA
cgcggaacccctatttgtttatttttctaaatacattcaaatatgtatccgctcatgagacaataaccctgataaatgcttcaataatattgaaaaaggaagagtatgagtattcaacatttccgtgtcgcccttattcccttttttgcggcattttgccttcctgtttttgctcacccagaaacgctggtgaaagtaaaagatgctgaagatcagttgggtgcacgagtgggttacatcgaactggatctcaacagcggtaagatccttgagagttttcgccccgaagaacgttttccaatgatgagcacttttaaagttctgctatgtggcgcggtattatcccgtattgacgccgggcaagagcaactcggtcgccgcatacactattctcagaatgacttggttgagtactcaccagtcacagaaaagcatcttacggatggcatgacagtaagagaattatgcagtgctgccataaccatgagtgataacactgcggccaacttacttctgacaacgatcggaggaccgaaggagctaaccgcttttttgcacaacatgggggatcatgtaactcgccttgatcgttgggaaccggagctgaatgaagccataccaaacgacgagcgtgacaccacgatgcctgtagcaatggcaacaacgttgcgcaaactattaactggcgaactacttactctagcttcccggcaacaattaatagactggatggaggcggataaagttgcaggaccacttctgcgctcggcccttccggctggctggtttattgctgataaatctggagccggtgagcgtgggtctcgcggtatcattgcagcactggggccagatggtaagccctcccgtatcgtagttatctacacgacggggagtcaggcaactatggatgaacgaaatagacagatcgctgagataggtgcctcactgattaagcattggtaactgtcagaccaagtttactcatatatactttagattgatttaaaacttcatttttaatttaaaaggatctaggtgaagatcctttttgataatctcatgaccaaaatcccttaacgtgagttttcgttccactgagcgtcagaccccgtagaaaagatcaaaggatcttc

SEQ ID NO: 24 - DNA, 806 bp, Artificial
  source 1..806: mol_type = other DNA
atcgagattttcaggagctaaggaagctaaaatggagaaaaaaatcactggatataccaccgttgatatatcccaatggcatcgtaaagaacattttgaggcatttcagtcagttgctcaatgtacctataaccagaccgttcagctggatattacggcctttttaaagaccgtaaagaaaaataagcacaagttttatccggcctttattcacattcttgcccgcctgatgaatgctcatccggaatttcgtatggcaatgaaagacggtgagctggtgatatgggatagtgttcacccttgttacaccgttttccatgagcaaactgaaacgttttcatcgctctggagtgaataccacgacgatttccggcagtttctacacatatattcgcaagatgtggcgtgttacggtgaaaacctggcctatttccctaaagggtttattgagaatatgtttttcgtctcagccaatccctgggtgagtttcaccagttttgatttaaacgtggccaatatggacaacttcttcgcccccgttttcaccatgggcaaatattatacgcaaggcgacaaggtgctgatgccgctggcgattcaggttcatcatgccgtttgtgatggcttccatgtcggcagaatgcttaatgaattacaacagtactgcgatgagtggcagggcggggcgtaatttgatatcgagctcgcttggactcctgttgatagatccagtaatgacctcagaactccatctggatttgttcagaacgctcggttgccgccgggcgttttttattggtgagaat

SEQ ID NO: 25 - DNA, 5951 bp, Artificial; identical to SEQ ID NO: 1
  source 1..5951: mol_type = other DNA

SEQ ID NO: 26 - DNA, 5603 bp, Artificial
  source 1..5603: mol_type = other DNA
caaattcaaattttaatttggaaattttgcgcccctccttctcgtgtactgtaaaaccaacaaacgaaatctcagttttctttttgatttctgcaatcgctttgtttaaaacatcgcgtttaaaaattgggaagtccgggtatttatattcgatgttcccgtctttatcaaaagtataggcaatcagttcttctttaagctcgtccacgctaatgataaaatagtttttttttttgaaattactataatgtttgcggatcagttgatacagtgatgaagaatactgtgacgacaggcgcaaggatgcagtcaataattgcgtggtaaatttgttctttttcccgataagactagaaatataaggctcaatagtacgcgtgaacttcagactcaagtagccctcgtcagggctgtaagcgatccactcaatgatattcaggtctaattcctccggggaatttttcgcagtgaatggcaagttcaactccttagcaagggcgatgatatcgtctccacgcaagctgatcttcgaggcgcccagcaatttgcctccctccttcagttgacggtaggccaaactaggagtaatttttgcaagcgccgctaagtcttcggcacgaatcttaaatacacgaccgcgttctaacggctccttactgtcaatgggggcaagggccatatacatcacgcgttttgctggtaaaggcagctgagctaaggtatgattaagctcattacgatgacgaatcttggtttttttattgacatccatcatcaccttcaaacgcatactcttcctttttcaatattattgaagcatttatcagggttattgtctcatgagcggatacatatttgaatgtatttagaaaaataaacaaataggggttccgcgtgcgtttctacaaactctttcggtccggaagatcctttgatcttttctacggggtctgacgctcagtggaacgaaaactcacgttaagggattttggtcatgaacaataaaactgtctgcttacataaacagtaatacaaggggtgttatgagccatattcaacgggaaacgtcttgctctaggccgcgattaaattccaacatggatgctgatttatatgggtataaatgggctcgcgataatgtcgggcaatcaggtgcgacaatctatcgattgtatgggaagcccgatgcgccagagttgtttctgaaacatggcaaaggtagcgttgccaatgatgttacagatgagatggtcagactaaactggctgacggaatttatgcctcttccgaccatcaagcattttatccgtactcctgatgatgcatggttactcaccactgcgatccccgggaaaacagcattccaggtattagaagaatatcctgattcaggtgaaaatattgttgatgcgctggcagtgttcctgcgccggttgcattcgattcctgtttgtaattgtccttttaacagcgatcgcgtatttcgtctcgctcaggcgcaatcacgaatgaataacggtttggttgatgcgagtgattttgatgacgagcgtaatggctggcctgttgaacaagtctggaaagaaatgcataaacttttgccattctcaccggattcagtcgtcactcatggtgatttctcacttgataaccttatttttgacgaggggaaattaataggttgtattgatgttggacgagtcggaatcgcagaccgataccaggatcttgccatcctatggaactgcctcggtgagttttctccttcattacagaaacggctttttcaaaaatatggtattgataatcctgatatgaataaattgcagtttcatttgatgctcgatgagtttttctaagaattaattcatgagcggatacatatttgaatgtatttagaaaaataaacaaataggggttccgcgcacatttccccgaaaagtgccacaggactgagcgtcaaccccgtagaaaagccccaactggggtaacctttgagttctctcagttgggggatcaaaggatcttcgtagacgatagatctactgactctgagttcgtagtagtgtacgtacggatatcagatctactgactctgagttcgtagtagtgtacgtacgtagtcagcacacaattgccattatacgcgcgtataatggactattgtgtgctgataaattggagatcggagctcgtacttcgcatgcatgcatgctggttgctgactaattgagatgcatgctttgcatacttctgcctgctggggagcctggggactttccacaccaatgcatgcatgctggttgctgactaattgagatgcatgctttgcatacttctgcctgctggggagcctggggactttccacaccaatgcatgcgtgcctatcaagatatttaaagaaaaaaaaattgtatcaactttctacaatctctttcagaagacagaagcagagggaatacttcctaaatcattcaactaggccagcattaccttaataccggaactagaaaatgacattacaagaaaagaaaacaacagaccaatatctctcatgaacaaagatacaaacattttcaacaaaatattagcaaaaagaatccaagaatgtatcaaaaaatatacaccacaaccaagtagaatttattccagatatgtaagggtggttcaacgtttgaaaatcaattaacgtaatttgtcccatcaacaggttaaagaagaaaatcacatggtcatattgatagacacagaaaaagcatttgacaaaatttaacacccattcatgatgcaatctctcagtaaactaggaatagaggaaaacttcctcagcttgaatgtaccttcctctcaattttgctatgaacctgaaactcctcttaaaaaataaagtttttcatttaaaaagaaaacaaaaaacatggaggagcgttgatgtatctcattttagaccaatcagctatggataggatccagacatgataagatacattgatgagtttggacaaaccacaactagaatgcagtgaaaaaaatgctttatttgtgaaatttgtgatgctattgctttatttgtaaccattataagctgcaataaacaagttaacaacaacaattgcattcattttatgtttcaggttcagggggaggtgtgggaggttttttaaagcaagtaaaacctctacaaatgtggtatggctgattatgatcnnnnnngagaccgtcgactctagagctagcgtacgtactaagctctcatgtttcacgtactaagctctcaagtttaacgtactaagctctcatgtttaacgaactaaaccctcatggctaacgtactaagctctcatggctaacgtactaagctctcatgtttcacgtactaagctctcatgtttgaacaataaaattaatataaatcagcaacttaaatagcctctaaggttttaagttttataagaaaaaaaagaatatataaggcttttaaagcttttaaggtttaacggttgtggacaacaagccagggatgtaacgcactgagaagcccttagagcctctcaaagcaattttgagtgacacaggaacacttaacggctgacannnnnngagaccgaattccctgcaggcgggagatgggggaggctaactgaaacacggaaggagacaataccggaaggaacccgcgctatgacggcaataaaaagacagaataaaacgcacgggtgttgggtcgtttgttcataaacgcggggttcggtcccagggctggcactctgtcgataccccaccgagaccccattgggaccaatacgcccgcgtttcttccttttccccaccccaacccccaagttcgggtgaaggcccagggctcgcagccaacgtcggggcggcaagccctgccatagccacctatcaagatatttaaagaaaaaaaaattgtatcaactttctacaatctctttcagaagacagaagcagagggaatacttcctaaatcattcaactaggccagcattaccttaataccggaactagaaaatgacattacaagaaaagaaaacaacagaccaatatctctcatgaacaaagatacaaacattttcaacaaaatattagcaaaaagaatccaagaatgtatcaaaaaatatacaccacaaccaagtagaatttattccagatatgtaagggtggttcaacgtttgaaaatcaattaacgtaatttgtcccatcaacaggttaaagaagaaaatcacatggtcatattgatagacacagaaaaagcatttgacaaaatttaacacccattcatgatgcaatctctcagtaaactaggaatagaggaaaacttcctcagcttgaatgtaccttcctctcaattttgctatgaacctgaaactcctcttaaaaaataaagtttttcatttaaaaagaaaacaaaaaacatggaggagcgttgatgtatctcattttagaccaatcagctatggatagatgcatgcatgctggttgctgactaattgagatgcatgctttgcatacttctgcctgctggggagcctggggactttccacaccaatgcatgcatgctggttgctgactaattgagatgcatgctttgcatacttctgcctgctggggagcctggggactttccacaccaatcgaaggaccatggtctgcgatcgtatcagcacacaatagtccattatacgcgcgtataatggcaattgtgtgctgaagttgacatctaggtaccgatatcgttgacatctagtacagttcagtacagtagtcactgacttgacactgacctcgagataacttcgtataatgtatgctatacgaagttatgcggccgcatcaaaggatcttctagggataacagggtaatgtcatctgggataacagggtaatgtcatctagggataacagggtatgtcatctgggataacagggtaatgtatctagggataacagggtaatgtcatctgggataacagggtaatgtcatctagggataacagggtatgtcatctgggataacagggtaatgtatctagggataacagggtaatgtcatctgggataacagggtaatgtcatctagggataacagggtatgtcatctgggataacagggtaatgtatctagggataacagggtaatgtcatctgggataacagggtaatgtcatctagggataacagggtatgtcatctgggataacagggtaatgtatctagggataacagggtaatgtcatctgggataacagggtaatgtcatctagggataacagggtatgtcatctgggataacagggtaatgtatcttgtatctagggataacagggtaatgaatgcgtcgagatactagtggatcccaaaaaacccctcaagacccgtttagaggccccaaggggttatgctagttattgctcagcggtggcagcagccaactcagcttcctttcgggcttttagcccttggcttttttgggcggaacggtttcatcgaacacttttaaaaatgccgcatcggcctccgacaagttcataaagaaagcctcgtcgtctttatctccactaaactcgtcctcatcaacga